European Patent Specification EP 3 207 056 B1, published June 25, 2025. Title: Norovirus antibodies. Applicant: Deutsches Krebsforschungszentrum Ruprecht-Karls-Universität. The sequence listing filed with the application follows.

SEQUENCE LISTING (12 sequences)

SEQ ID NO: 1 - protein, 7 aa, Norovirus
  VARIANT (4)..(4): Xaa is any amino acid, preferably Q or P
  VARIANT (7)..(7): Xaa is any amino acid, preferably T or S
WVNXFYX

SEQ ID NO: 2 - protein, 12 aa, Norovirus
  VARIANT (2)..(5): Xaa is any amino acid
  VARIANT (9)..(9): Xaa is any amino acid, preferably  Q or P
  VARIANT (12)..(12): Xaa is any amino acid, preferably T or S
FXXXXWVNXFYX

SEQ ID NO: 3 - protein, 60 aa, Norovirus
  VARIANT (1)..(1): Xaa is a non-charged amino acid, preferably L, P, M, Q, or N
  VARIANT (2)..(53): Xaa is a any amino acid
  VARIANT (57)..(57): Xaa is any amino acid, preferably Q or P
  VARIANT (60)..(60): Xaa is any amino acid, preferably, T or S
XXXXXXXXXXXXXXXXXXXXXXXXXXXXXXXXXXXXXXXXXXXXXXXXXXXXXWVNXFYX

SEQ ID NO: 4 - protein, 60 aa, Norovirus
  VARIANT (1)..(1): Xaa is a non-charged amino acid, preferably L, P, M, Q, or N
  VARIANT (2)..(53): Xaa is a non-charged amino acid, preferably L, P, M, Q, or N
  VARIANT (2)..(48): Xaa is any amino acid
  VARIANT (50)..(53): Xaa is any amino acid
  VARIANT (57)..(57): Xaa is any amino acid, preferably Q or P
  VARIANT (60)..(60): Xaa is any amino acid, preferably T or S
XXXXXXXXXXXXXXXXXXXXXXXXXXXXXXXXXXXXXXXXXXXXXXXXFXXXXWVNXFYX

SEQ ID NO: 5 - DNA, 381 bp, Artificial
  synthetic sb-AB from Lama pacos
gatgtgcagctggtggagtctgggggaggcttggtgcagcctggggggtctctgagactctcctgtgcagcctctggaagcatcttcagtatctatgccatgggctggtaccgccaggctccagggaagcagcgcgagttggtcgcttctattagtagtggtggtggcacaaactatgcagactccgtgaagggccgattcaccatctccggagacaacgccaagaacacggtgtatctgcaaatgaacagcctgaaacctgaggacacggccgtctattactgtaaaagagaagactatagcgcctatgcgcccccgagtggttcccggggccgggggacccaggtcaccgtctcctcacaccaccatcaccatcactaa

SEQ ID NO: 6 - protein, 8 aa, Lama pacos
GSIFSIYA

SEQ ID NO: 7 - protein, 8 aa, Lama pacos
ISSGGGTN

SEQ ID NO: 8 - protein, 14 aa, Lama pacos
KREDYSAYAPPSGS

SEQ ID NO: 9 - protein, 135 aa, Artificial
  synthetic sb-AB from Lama pacos
DVQLVESGGGLVQPGGSLRLSCAASGSIFSIYAMGWYRQAPGKQRELVASISSGGGTNYADSVKGRFTISGDNAKNTVYLQMNSLKPEDTAVYYCKREDYSAYAPPSGSRGRGTQVTVSSGRYPYDVPDYGSGRA

SEQ ID NO: 10 - protein, 7 aa, Norovirus
WVNQFYT

SEQ ID NO: 11 - protein, 7 aa, Norovirus
WVNQFYS

SEQ ID NO: 12 - protein, 7 aa, Norovirus
WVNPFYT